European Patent Application EP 4 471 050 A1, published December 4, 2024. Title: POLYETHYLENE GLYCOL-MODIFIED FORM OF KININ OR DERIVATIVE THEREOF AND PHARMACEUTICAL USE THEREOF. Applicant: ZonHon Biopharma Institute, Inc. Application EP. The sequence listing filed with the application follows.

SEQUENCE LISTING (17 sequences)

SEQ ID NO: 1 - protein, 10 aa, Homo sapiens
KRPPGFSPFR

SEQ ID NO: 2 - protein, 10 aa, synthetic construct
  SITE 6: note = beta-2-thienylalanine
KRPPGXSPFR

SEQ ID NO: 3 - protein, 9 aa, synthetic construct
  SITE 5: note = beta-2-thienylalanine
RPPGXSPFR

SEQ ID NO: 4 - protein, 10 aa, synthetic construct
KRPPGHSPFR

SEQ ID NO: 5 - protein, 10 aa, synthetic construct
KRPPGFSPHR

SEQ ID NO: 6 - protein, 9 aa, synthetic construct
  SITE 6: note = beta-2-thienylalanine
KRPPGXSPF

SEQ ID NO: 7 - protein, 11 aa, synthetic construct
  SITE 6: note = beta-2-thienylalanine
KRPPGXSPFRR

SEQ ID NO: 8 - protein, 10 aa, synthetic construct
  SITE 6: note = beta-2-thienylalanine
  SITE 9: note = beta-2-thienylalanine
KRPPGXSPXR

SEQ ID NO: 9 - protein, 7 aa, synthetic construct
  SITE 3: note = beta-2-thienylalanine
PGXSPFR

SEQ ID NO: 10 - protein, 5 aa, synthetic construct
  SITE 1: note = beta-2-thienylalanine
XSPFR

SEQ ID NO: 11 - protein, 4 aa, synthetic construct
SPFR

SEQ ID NO: 12 - protein, 11 aa, synthetic construct
  SITE 7: note = beta-2-thienylalanine
KRRPPGXSPFR

SEQ ID NO: 13 - protein, 19 aa, synthetic construct
  SITE 6: note = beta-2-thienylalanine
  SITE 15: note = beta-2-thienylalanine
KRPPGXSPFRRPPGXSPFR

SEQ ID NO: 14 - protein, 11 aa, synthetic construct
  SITE 7: note = beta-2-thienylalanine
CRRPPGXSPFR

SEQ ID NO: 15 - protein, 20 aa, synthetic construct
  SITE 6: note = beta-2-thienylalanine
  SITE 16: note = beta-2-thienylalanine
KRPPGXSPFRKRPPGXSPFR

SEQ ID NO: 16 - protein, 10 aa, synthetic construct
  SITE 6: note = beta-2-thienylalanine
CRPPGXSPFR

SEQ ID NO: 17 - protein, 12 aa, synthetic construct
  SITE 8: note = beta-2-thienylalanine
CRRRPPGXSPFR